European Patent Application EP 4 450 616 A2, published October 23, 2024. Title: The novel monoclonal antibodies to programmed death 1 (PD-1). Applicant: CStone Pharmaceuticals. The sequence listing filed with the application follows.

SEQUENCE LISTING (33 sequences)

SEQ ID NO: 1 - protein, 115 aa, synthetic construct
  REGION 1..115: note = Variable region of a heavy chain
QVQLVQSGAEVKKPGSSVKVSCKASGFTFTTYYISWVRQAPGQGLEYLGYINMGSGGTNYNEKFKGRVTITADKSTSTAYMELSSLRSEDTAVYYCAILGYFDYWGQGTMVTVSS

SEQ ID NO: 2 - protein, 115 aa, synthetic construct
  REGION 1..115: note = Variable region of a heavy chain
QVQLVQSGAEVKKPGSSVKVSCKASGFTFTTYYISWVRQAPGQGLEYLGYINMGSGGTNYNEKFKGRVTITADKSTSTAYMELSSLRSEDTAVYYCAIIGYFDYWGQGTMVTVSS

SEQ ID NO: 3 - protein, 112 aa, synthetic construct
  REGION 1..112: note = Variable region of a light chain
DVVMTQSPLSLPVTLGQPASISCRSSQSLLDSDGGTYLYWFQQRPGQSPRRLIYLVSTLGSGVPDRFSGSGSGTDFTLKISRVEAEDVGVYYCMQLTHWPYTFGQGTKLEIK

SEQ ID NO: 4 - protein, 112 aa, synthetic construct
  REGION 1..112: note = Variable region of a light chain
DVVMTQSPLSLPVTLGQPASISCRSSQSLLDSDGSTYLYWFQQRPGQSPRRLIYLVSTLGSGVPDRFSGSGSGTDFTLKISRVEAEDVGVYYCMQLTHWPYTFGQGTKLEIK

SEQ ID NO: 5 - protein, 112 aa, synthetic construct
  REGION 1..112: note = Variable region of a light chain
DVVMTQSPLSLPVTLGQPASISCRSSQSLLDSDGATYLYWFQQRPGQSPRRLIYLVSTLGSGVPDRFSGSGSGTDFTLKISRVEAEDVGVYYCMQLTHWPYTFGQGTKLEIK

SEQ ID NO: 6 - protein, 112 aa, synthetic construct
  REGION 1..112: note = Variable region of a light chain
DVVMTQSPLSLPVTLGQPASISCRSSQSLLDSDGNTYLYWFQQRPGQSPRRLIYLVSTLGSGVPDRFSGSGSGTDFTLKISRVEAEDVGVYYCMQLTHWPYTFGQGTKLEIK

SEQ ID NO: 7 - protein, 112 aa, synthetic construct
  REGION 1..112: note = Variable region of a light chain
DVVMTQSPLSLPVTLGQPASISCRSSQSLLDSDGNTYLYWFQQRPGQSPRRLIYLVSTLGSGVPDRFSGSGSGTDFTLKISRVEAEDVGVYYCMQLTHAPYTFGQGTKLEIK

SEQ ID NO: 8 - protein, 112 aa, synthetic construct
  REGION 1..112: note = Variable region of a light chain
DVVMTQSPLSLPVTLGQPASISCRSSQSLLDSDGQTYLYWFQQRPGQSPRRLIYLVSTLGSGVPDRFSGSGSGTDFTLKISRVEAEDVGVYYCMQLTHEPYTFGQGTKLEIK

SEQ ID NO: 9 - protein, 112 aa, synthetic construct
  REGION 1..112: note = Variable region of a light chain
DVVMTQSPLSLPVTLGQPASISCRSSQSLLDSDGQTYLYWFQQRPGQSPRRLIYLVSTLGSGVPDRFSGSGSGTDFTLKISRVEAEDVGVYYCMQLTHENYTFGQGTKLEIK

SEQ ID NO: 10 - protein, 5 aa, synthetic construct
  REGION 1..5: note = CDR1 of a heavy chain
TYYIS

SEQ ID NO: 11 - protein, 17 aa, synthetic construct
  REGION 1..17: note = CDR2 of a heavy chain
YINMGSGGTNYNEKFKG

SEQ ID NO: 12 - protein, 6 aa, synthetic construct
  REGION 1..6: note = CDR3 of a heavy chain
LGYFDY

SEQ ID NO: 13 - protein, 6 aa, synthetic construct
  REGION 1..6: note = CDR3 of a heavy chain
IGYFDY

SEQ ID NO: 14 - protein, 16 aa, synthetic construct
  REGION 1..16: note = CDR1 of a light chain
RSSQSLLDSDGGTYLY

SEQ ID NO: 15 - protein, 16 aa, synthetic construct
  REGION 1..16: note = CDR1 of a light chain
RSSQSLLDSDGSTYLY

SEQ ID NO: 16 - protein, 16 aa, synthetic construct
  REGION 1..16: note = CDR1 of a light chain
RSSQSLLDSDGATYLY

SEQ ID NO: 17 - protein, 16 aa, synthetic construct
  REGION 1..16: note = CDR1 of a light chain
RSSQSLLDSDGNTYLY

SEQ ID NO: 18 - protein, 16 aa, synthetic construct
  REGION 1..16: note = CDR1 of a light chain
RSSQSLLDSDGQTYLY

SEQ ID NO: 19 - protein, 7 aa, synthetic construct
  REGION 1..7: note = CDR2 of a light chain
LVSTLGS

SEQ ID NO: 20 - protein, 9 aa, synthetic construct
  REGION 1..9: note = CDR3 of a light chain
MQLTHENYT

SEQ ID NO: 21 - protein, 9 aa, synthetic construct
  REGION 1..9: note = CDR3 of a light chain
MQLTHWPYT

SEQ ID NO: 22 - protein, 9 aa, synthetic construct
  REGION 1..9: note = CDR3 of a light chain
MQLTHAPYT

SEQ ID NO: 23 - protein, 9 aa, synthetic construct
  REGION 1..9: note = CDR3 of a light chain
MQLTHEPYT

SEQ ID NO: 24 - protein, 288 aa, Homo sapiens
  REGION 1..288: note = PD-1
MQIPQAPWPVVWAVLQLGWRPGWFLDSPDRPWNPPTFSPALLVVTEGDNATFTCSFSNTSESFVLNWYRMSPSNQTDKLAAFPEDRSQPGQDCRFRVTQLPNGRDFHMSVVRARRNDSGTYLCGAISLAPKAQIKESLRAELRVTERRAEVPTAHPSPSPRPAGQFQTLVVGVVGGLLGSLVLLVWVLAVICSRAARGTIGARRTGQPLKEDPSAVPVFSVDYGELDFQWREKTPEPPVPCVPEQTEYATIVFPSGMGTSSPARRGSADGPRSAQPLRPEDGHCSWPL

SEQ ID NO: 25 - protein, 11 aa, synthetic construct
  REGION 1..11: note = VKCDR1
LDSDGGTYLYW

SEQ ID NO: 26 - protein, 11 aa, synthetic construct
  REGION 1..11: note = VKCDR1
LDSDGSTYLYW

SEQ ID NO: 27 - protein, 11 aa, synthetic construct
  REGION 1..11: note = VKCDR1
LDSDGATYLYW

SEQ ID NO: 28 - protein, 11 aa, synthetic construct
  REGION 1..11: note = VKCDR1
LDSDGNTYLYW

SEQ ID NO: 29 - protein, 11 aa, synthetic construct
  REGION 1..11: note = VKCDR1
LDSDGQTYLYW

SEQ ID NO: 30 - protein, 12 aa, synthetic construct
  REGION 1..12: note = VKCDR3
MQLTHWPYTFGQ

SEQ ID NO: 31 - protein, 12 aa, synthetic construct
  REGION 1..12: note = VKCDR3
MQLTHENYTFGQ

SEQ ID NO: 32 - protein, 12 aa, synthetic construct
  REGION 1..12: note = VKCDR3
MQLTHEPYTFGQ

SEQ ID NO: 33 - protein, 12 aa, synthetic construct
  REGION 1..12: note = VKCDR3
MQLTHAPYTFGQ